European Patent Application EP 4 632 381 A1, published October 15, 2025. Title: METHOD AND KIT FOR PREDICTING EFFICACY OF TREATMENT WITH IMMUNOTHERAPEUTIC AGENT ON PATIENT WITH MUCOSAL LESION. Applicant: NIHON UNIVERSITY. Application JP PCT/JP2024/001302, filed January 18, 2024. The sequence listing filed with the application follows.

SEQUENCE LISTING (8 sequences)

SEQ ID NO: 1 - protein, 98 aa, Human papillomavirus type 16
MHGDTPTLHEYMLDLQPETTDLYCYEQLNDSSEEEDEIDGPAGQAEPDRAHYNIVTFCCKCDSTLRLCVQSTHVDIRTLEDLLMGTLGIVCPICSQKP

SEQ ID NO: 2 - protein, 98 aa, Human papillomavirus type 16
MHGDTPTLHEYMLDLQPETTGLYGYGQLNDSSEEEDEIDGPAGQAEPDRAHYNIVTFCCKCDSTLRLCVQSTHVDIRTLEDLLMGTLGIVCPICSQKP

SEQ ID NO: 3 - DNA, 23 bp, synthetic construct
  source 1..23: mol_type = other DNA
aagtgtgactctacgcttcggtt

SEQ ID NO: 4 - DNA, 22 bp, synthetic construct
  source 1..22: mol_type = other DNA
gcccattaacaggtcttccaaa

SEQ ID NO: 5 - DNA, 28 bp, synthetic construct
  source 1..28: mol_type = other DNA
aggagcgacccggaaagttaccacagtt

SEQ ID NO: 6 - DNA, 18 bp, synthetic construct
  source 1..18: mol_type = other DNA
aggcatgcagatcccaca

SEQ ID NO: 7 - DNA, 20 bp, synthetic construct
  source 1..20: mol_type = other DNA
cctgtctggggagtctaaga

SEQ ID NO: 8 - DNA, 19 bp, synthetic construct
  source 1..19: mol_type = other DNA
tctgggcggtgctacaact